European Patent Application EP 4 177 267 A1, published May 10, 2023. Title: ANTI-SURROGATE LIGHT CHAIN ANTIBODIES. Applicant: Children's Health Care d/b/a Children's Minnesota. Application EP. The sequence listing filed with the application follows.

SEQUENCE LISTING (69 sequences)

SEQ ID NO: 1 - protein, 145 aa, Homo sapiens
MSWAPVLLMLFVYCTGCGPQPVLHQPPAMSSALGTTIRLTCTLRNDHDIGVYSVYWYQQRPGHPPRFLLRYFSQSDKSQGPQVPPRFSGSKDVARNRGYLSISELQPEDEAMYYCAMGARSSEKEEREREWEEEMEPTAARTRVP

SEQ ID NO: 2 - protein, 142 aa, Mus musculus
MAWTSVLLMLLAHLTGCGPQPMVHQPPSASSSLGATIRLSCTLSNDHNIGIYSIYWYQQRPGHPPRFLLRYFSHSDKHQGPDIPPRFSGSKDTARNLGYLSISELQPEDEAVYYCAVGLRSHEKKRMEREWEGEKSYTDLGS

SEQ ID NO: 3 - protein, 171 aa, Mus musculus
MAWTSVLLMLLAHLTGKGTLGVQGFLAPPVALLCPSDGHASIFSGCGPQPMVHQPPSASSSLGATIRLSCTLSNDHNIGIYSIYWYQQRPGHPPRFLLRYFSHSDKHQGPDIPPRFSGSKDTARNLGYLSISELQPEDEAVYYCAVGLRSHEKKRMEREWEGEKSYTDLGS

SEQ ID NO: 4 - protein, 123 aa, Homo sapiens
MACRCLSFLLMGTFLSVSQTVLAQLDALLVFPGQVAQLSCTLSPQHVTIRDYGVSWYQQRAGSAPRYLLYYRSEEDHHRPADIPDRFSAAKDEAHNACVLTISPVQPEDDADYYCSVGYGFSP

SEQ ID NO: 5 - protein, 119 aa, Homo sapiens
MSWAPVLLMLFVYCTGCGPQPVLHQPPAMSSALGTTIRLTCTLRNDHDIGVYSVYWYQQRPGHPPRFLLRYFSQSDKSQGPQVPPRFSGSKDVARNRGYLSISELQPEDEAMYYCAMGA

SEQ ID NO: 6 - protein, 146 aa, synthetic construct
  REGION 1..146: note = Description of Artificial Sequence: Synthetic polypeptide
METDTLLLWVLLLWVPGSTGQPVLHQPPAMSSALGTTIRLTCTLRNDHDIGVYSVYWYQQRPGHPPRFLLRYFSQSDKSQGPQVPPRFSGSKDVARNRGYLSISELQPEDEAMYYCAMGARSSEKEEREREWEEEMEPTAARTRVP

SEQ ID NO: 7 - protein, 209 aa, Homo sapiens
MKLRVGQTLGTIPRQCEVLLLLLLLGLVDGVHHILSPSSAERSRAVGPGASVGSNRPSLWALPGRLLFQIIPRGAGPRCSPHRLPSKPQFWYVFGGGTQLTILGQPKSDPLVTLFLPSLKNLQPTRPHVVCLVSEFYPGTLVVDWKVDGVPVTQGVETTQPSKQTNNKYMVSSYLTLISDQWMPHSRYSCRVTHEGNTVEKSVSPAECS

SEQ ID NO: 8 - protein, 213 aa, Homo sapiens
MRPGTGQGGLEAPGEPGPNLRQRWPLLLLGLAVVTHGLLRPTAASQSRALGPGAPGGSSRSSLRSRWGRFLLQRGSWTGPRCWPRGFQSKHNSVTHVFGSGTQLTVLSQPKATPSVTLFPPSSEELQANKATLVCLMNDFYPGILTVTWKADGTPITQGVEMTTPSKQSNNKYAASSYLSLTPEQWRSRRSYSCQVMHEGSTVEKTVAPAECS

SEQ ID NO: 9 - protein, 158 aa, Homo sapiens
MRPGTGQGGLEAPGEPGPNLRQRWPLLLLGLAVVTHGSVTHVFGSGTQLTVLSQPKATPSVTLFPPSSEELQANKATLVCLMNDFYPGILTVTWKADGTPITQGVEMTTPSKQSNNKYAASSYLSLTPEQWRSRRSYSCQVMHEGSTVEKTVAPAECS

SEQ ID NO: 10 - protein, 141 aa, synthetic construct
  REGION 1..141: note = Description of Artificial Sequence: Synthetic polypeptide
METDTLLLWVLLLWVPGSTGSVTHVFGSGTQLTVLSQPKATPSVTLFPPSSEELQANKATLVCLMNDFYPGILTVTWKADGTPITQGVEMTTPSKQSNNKYAASSYLSLTPEQWRSRRSYSCQVMHEGSTVEKTVAPAECS

SEQ ID NO: 11 - DNA, 711 bp, Homo sapiens
  source 1..711: mol_type = other DNA
  CDS 8..547: protein_id = 68; translation = MVLQTQVFISLLLWISGAYGDIVMTQSPDSLAVSLGERATINCKSSQSVLYSSNNKNYLAWYQQKPGQPPKLLIYWASTRESGVPDRFSGSGSGTDFTLTISSLQAEDVAVYYCQQYYSTPPTVLQPRTQTSSPYAGPVGLCCSSCFLCTQPPTCMLPLCVGEVTLLIYSLEGLQGPGLN
cagcaagatggtgttgcagacccaggtcttcatttctctgttgctctggatctctggtgcctacggggacatcgtgatgacccagtctccagactccctggctgtgtctctgggcgagagggccaccatcaactgcaagtccagccagagtgttttatacagctccaacaataagaactacttagcttggtaccagcagaaaccaggacagcctcctaagctgctcatttactgggcatctacccgggaatccggggtccctgaccgattcagtggcagcgggtctgggacagatttcactctcaccatcagcagcctgcaggctgaagatgtggcagtttattactgtcagcaatattatagtactcctcccacagtgcttcagcctcgaacacaaacctcctccccatacgctgggccagtaggtctttgctgcagcagctgcttcctctgcacacagcccccaacatgcatgcttcctctgtgtgttggggaggtcactctcttgatttattcgttggagggtttgcagggcccaggattaaattaagagacttgacttttgctggatctctttttgtagaagattattaaagcaaaatgttgtaaagatcccttagagacattgtcaggagtttttgtgttacaggaacctgcatgtttcacatggacacatcacatgaccgagccaaatagatttatctttactct

SEQ ID NO: 12 - protein, 180 aa, Homo sapiens
MVLQTQVFISLLLWISGAYGDIVMTQSPDSLAVSLGERATINCKSSQSVLYSSNNKNYLAWYQQKPGQPPKLLIYWASTRESGVPDRFSGSGSGTDFTLTISSLQAEDVAVYYCQQYYSTPPTVLQPRTQTSSPYAGPVGLCCSSCFLCTQPPTCMLPLCVGEVTLLIYSLEGLQGPGLN

SEQ ID NO: 13 - protein, 103 aa, Homo sapiens
DIQMTQSPSSVSASVGDRVTITCRASQGISSWLAWYQQKPGKAPKLLIYAASSLQSGVPSRFSGSGSGTDFTLTISSLQPEDFATYYCQQANSFPPTVLPTRT

SEQ ID NO: 14 - protein, 103 aa, Homo sapiens
DIQMTQSPSSLSASVGDRVTITCRASQGISNYLAWFQQKPGKAPKSLIYAASSLQSGVPSRFSGSGSGTDFTLTISSLQPEDFATYYCQQYNSYPPTVLHTQT

SEQ ID NO: 15 - protein, 110 aa, Homo sapiens
DIQMTQSPSSLSASVGDRVTITCRASQGIRNDLGWYQQKPGKAPKRLIYAASSLQSGVPSRFSGSGSGTEFTLTISSLQPEDFATYYCLQHNSYPPTVLHTRTTPREADV

SEQ ID NO: 16 - protein, 98 aa, Homo sapiens
DIQMTQSPSSLSASVGDRVTITCQASQDISNYLNWYQQKPGKAPKLLIYDASNLETGVPSRFSGSGSGTDFTFTISSLQPEDIATYYCQQYDNLPPTV

SEQ ID NO: 17 - protein, 101 aa, Homo sapiens
DIQMIQSPSFLSASVGDRVSIICWASEGISSNLAWYLQKPGKSPKLFLYDAKDLHPGVSSRFSGRGSGTDFTLTIISLKPEDFAAYYCKQDFSYPPTGLQA

SEQ ID NO: 18 - protein, 136 aa, Homo sapiens
DIVMTQSPLSLPVTPGEPASISCRSSQSLLHGSNGYNYLDWYLQKPGQSPQLLIYLGSNRASGVPDRFSGSGSGTDFTLKISRVEAEDVGVYYCMQALQTPPTVVQPLTETSSWGCPVAHMCCLSGEQLSRVSESA

SEQ ID NO: 19 - protein, 106 aa, Homo sapiens
DVVMTQSPLSLPVTLGQPASISCRSSQSLVYSDGNTYLNWFQQRPGQSFRRLIYKVSNRDSGVPDRFSGSGSGTDFTLKISRVEAEDVGVYYCMQGTHWPPTVVQP

SEQ ID NO: 20 - protein, 132 aa, Homo sapiens
EIVLTQSPATLSLSPGERATLSCRASQSVSSYLAWYQQKPGQAPRLLIYDASNRATGIPARFSGSGSGTDFTLTISSLEPEDFAVYYCQQRSNWPPTVIPHETKTPTRPSVFTRLLYQLLPLQTASGVATQC

SEQ ID NO: 21 - protein, 118 aa, Homo sapiens
EIVLTQSPATLSLSPGERATLSCRASQGVSSYLAWYQQKPGQAPRLLIYDASNRATGIPARFSGSGPGTDFTLTISSLEPEDFAVYYCQQRSNWHPTVIPHETKTPTRPSVFTRLLYQ

SEQ ID NO: 22 - protein, 115 aa, Homo sapiens
ETTLTQSPAFMSATPGDKVNISCKASQDIDDDMNWYQQKPGEAAIFIIQEATTLVPGIPPRFSGSGYGTDFTLTINNIESEDAAYYFCLQHDNFPLTVIHPVQKPPSSLSGIASA

SEQ ID NO: 23 - protein, 158 aa, Homo sapiens
DVVMTQSPAFLSVTPGEKVTITCQASEGIGNYLYWYQQKPDQAPKLLIKYASQSISGVPSRFSGSGSGTDFTFTISSLEAEDAATYYCQQGNKHPHTVLQPKTKISSAWRNRETEQYPVFMILAGAVGEIIYQIPSHMAHSAELTPKSQCLTLSSLPT

SEQ ID NO: 24 - protein, 103 aa, Homo sapiens
DIVLTQSPASLAVSPGQRATITCRASESVSFLGINLIHWYQQKPGQPPKLLIYQASNKDTGVPARFSGSGSGTDFTLTINPVEANDTANYYCLQSKNFPPTVL

SEQ ID NO: 25 - DNA, 408 bp, Homo sapiens
  source 1..408: mol_type = other DNA
  CDS 1..405: protein_id = 69; translation = VRRVFVQQDNGELTLWWTFGQGTKVEIKRTVAAPSVFIFPPSDEQLKSGTASVVCLLNNFYPREAKVQWKVDNALQSGNSQESVTEQDSKDSTYSLSSTLTLSKADYEKHKLYACEVTHQGLSSPVTKSFNRGEC
gtgagaagggtttttgttcagcaagacaatggagagctcacactgtggtggacgttcggccaagggaccaaggtggaaatcaaacgaactgtggctgcaccatctgtcttcatcttcccgccatctgatgagcagttgaaatctggaactgcctctgttgtgtgcctgctgaataacttctatcccagagaggccaaagtacagtggaaggtggataacgccctccaatcgggtaactcccaggagagtgtcacagagcaggacagcaaggacagcacctacagcctcagcagcaccctgacgctgagcaaagcagactacgagaaacacaaactctacgcctgcgaagtcacccatcagggcctgagctcgcccgtcacaaagagcttcaacaggggagagtgttag

SEQ ID NO: 26 - protein, 135 aa, Homo sapiens
VRRVFVQQDNGELTLWWTFGQGTKVEIKRTVAAPSVFIFPPSDEQLKSGTASVVCLLNNFYPREAKVQWKVDNALQSGNSQESVTEQDSKDSTYSLSSTLTLSKADYEKHKLYACEVTHQGLSSPVTKSFNRGEC

SEQ ID NO: 27 - protein, 119 aa, Homo sapiens
WTFGQGTKVEIKRTVAAPSVFIFPPSDEQLKSGTASVVCLLNNFYPREAKVQWKVDNALQSGNSQESVTEQDSKDSTYSLSSTLTLSKADYEKHKLYACEVTHQGLSSPVTKSFNRGEC

SEQ ID NO: 28 - protein, 119 aa, Homo sapiens
YTFGQGTKLEIKRTVAAPSVFIFPPSDEQLKSGTASVVCLLNNFYPREAKVQWKVDNALQSGNSQESVTEQDSKDSTYSLSSTLTLSKADYEKHKLYACEVTHQGLSSPVTKSFNRGEC

SEQ ID NO: 29 - protein, 119 aa, Homo sapiens
FTFGPGTKVDIKRTVAAPSVFIFPPSDEQLKSGTASVVCLLNNFYPREAKVQWKVDNALQSGNSQESVTEQDSKDSTYSLSSTLTLSKADYEKHKLYACEVTHQGLSSPVTKSFNRGEC

SEQ ID NO: 30 - protein, 119 aa, Homo sapiens
LTFGGGTKVEIKRTVAAPSVFIFPPSDEQLKSGTASVVCLLNNFYPREAKVQWKVDNALQSGNSQESVTEQDSKDSTYSLSSTLTLSKADYEKHKLYACEVTHQGLSSPVTKSFNRGEC

SEQ ID NO: 31 - protein, 119 aa, Homo sapiens
ITFGQGTRLEIKRTVAAPSVFIFPPSDEQLKSGTASVVCLLNNFYPREAKVQWKVDNALQSGNSQESVTEQDSKDSTYSLSSTLTLSKADYEKHKLYACEVTHQGLSSPVTKSFNRGEC

SEQ ID NO: 32 - protein, 154 aa, synthetic construct [sequence omitted]

SEQ ID NO: 33 - protein, 138 aa, synthetic construct
  REGION 1..138: note = Description of Artificial Sequence: Synthetic polypeptide
METDTLLLWVLLLWVPGSTGWTFGQGTKVEIKRTVAAPSVFIFPPSDEQLKSGTASVVCLLNNFYPREAKVQWKVDNALQGNSQESVTEQDSKDSTYSLSSTLTLSKADYEKHKLYACEVTHQGLSSPVTKSFNRGEC

SEQ ID NO: 34 - protein, 132 aa, synthetic construct
  REGION 1..132: note = Description of Artificial Sequence: Synthetic polypeptide
METDTLLLWVLLLWVPGSTGTKVEIKRTVAAPSVFIFPPSDEQLKSGTASVVCLLNNFYPREAKVQWKVDNALQGNSQESVTEQDSKDSTYSLSSTLTLSKADYEKHKLYACEVTHQGLSSPVTKSFNRGEC

SEQ ID NO: 35 - protein, 243 aa, synthetic construct
  REGION 1..243: note = Description of Artificial Sequence: Synthetic polypeptide
METDTLLLWVLLLWVPGSTGQPVLHQPPAMSSALGTTIRLTCTLRNDHDIGVYSVYWYQQRPGHPPRFLLRYFSQSDKSQGPQVPPRFSGSKDVARNRGYLSISELQPEDEAMYYCAMGARSSVTHVFGSGTQLTVLSQPKATPSVTLFPPSSEELQANKATLVCLMNDFYPGILTVTWKADGTPITQGVEMTTPSKQSNNKYAASSYLSLTPEQWRSRRSYSCQVMHEGSTVEKTVAPAECS

SEQ ID NO: 36 - protein, 216 aa, synthetic construct
  REGION 1..216: note = Description of Artificial Sequence: Synthetic polypeptide
ALDIQLTQSPSFLSASVGDRVTITCRASQGINTWLAWYQQKPGKAPKLLIYAASTLQSGVPSRFSGSGSGTEFTLTISSLQPEDFATYYCQQLNSYPLTFGGGTKVEIKRTVAAPSVFIFPPSDEQLKSGTASVVCLLNNFYPREAKVQWKVDNALQSGNSQESVTEQDSKDSTYSLSSTLTLSKADYEKHKVYACEVTHQGLSSPVTKSFNRGEC

SEQ ID NO: 37 - protein, 216 aa, synthetic construct
  REGION 1..216: note = Description of Artificial Sequence: Synthetic polypeptide
ALDIQLTQSPSFLSASVGDRVTITCRASQGISTDLAWYQQKPGKAPKLLIYDASSLESGVPSRFSGSGSGTEFTLTISSLQPEDFATYYCQQANSFPFTFGGGTKVEIKRTVAAPSVFIFPPSDEQLKSGTASVVCLLNNFYPREAKVQWKVDNALQSGNSQESVTEQDSKDSTYSLSSTLTLSKADYEKHKVYACEVTHQGLSSPVTKSFNRGEC

SEQ ID NO: 38 - protein, 217 aa, synthetic construct
  REGION 1..217: note = Description of Artificial Sequence: Synthetic polypeptide
ALEIVLTQSPGTLSLSPGERATLSCRASQSVSSSYLAWYQQKPGQAPRLLIYGASSRATGIPDRFSGSGSGTDFTLTISRLEPEDFAVYYCQQYGNSPRTFGGGTKVEIKRTVAAPSVFIFPPSDEQLKSGTASVVCLLNNFYPREAKVQWKVDNALQRGNSQESVTEQDSKDSTYSLSSTLTLSKADYEKHKVYACEVTHQGLSSPVTKSFNRGEC

SEQ ID NO: 39 - protein, 216 aa, synthetic construct
  REGION 1..216: note = Description of Artificial Sequence: Synthetic polypeptide
ALDIQMTQSPSSLSASVGDRVTITCRASQGISNYLAWFQQKPGKAPKSLIYAASSLQSGVPSRFSGSGSGTDFTLTISSLQPEDFATYYCQQYNSYPLTFGGGTKVEIKRTVAAPSVFIFPPSDEQLKSGTASVVCLLNNFYPREAKVQWKVDNALQSGNSQESVTEQDSKDSTYSLSSTLTLSKADYEKHKVYACEVTHQGLSSPVTKSFNRGEC

SEQ ID NO: 40 - protein, 216 aa, synthetic construct
  REGION 1..216: note = Description of Artificial Sequence: Synthetic polypeptide
ALDIQMTQSPSSLSASVGDRVTITCRASQGISNYLAWFQQKPGKAPKSLIYAASTLESGVPSRFSGSGSGTDFTLTISSLQPEDFATYYCQQYNSYPLTFGGGTKVEIKRTVAAPSVFIFPPSDEQLKSGTASVVCLLNNFYPREAKVQWKVDNALQSGNSQESVTEQDSKDSTYSLSSTLTLSKADYEKHKVYACEVTHQGLSSPVTKSFNRGEC

SEQ ID NO: 41 - protein, 216 aa, synthetic construct
  REGION 1..216: note = Description of Artificial Sequence: Synthetic polypeptide
ALDIQLTQSPSFLSASVGDRVTITCRASQGIGNDLNWYQQKPGKAPKLLIYDASSLESGVPSRFSGSGSGTEFTLTISSLQPEDFATYYCQQADSWPLTFGGGTKVEIKRTVAAPSVFIFPPSDEQLKSGTASVVCLLNNFYPREAKVQWKVDNALQSGNSQESVTEQDSKDSTYSLSSTLTLSKADYEKHKVYACEVIHQGLSSPVTKSFNRGEC

SEQ ID NO: 42 - protein, 216 aa, synthetic construct
  REGION 1..216: note = Description of Artificial Sequence: Synthetic polypeptide
ALDIQLTQSPSFLSASVGDRVTITCRASQGISTDLNWYQQKPGKAPKLLIYAASNLESGVPSRFSGSGSGTEFTLTISSLQPEDFATYYCQQSYNWPYTFGGGTKVEIKRTVAAPSVFIFPPSDEQLKSGTASVVCLLNNFYPREAKVQWKVDNALQSGNSQESVTEQDSKDSTYSLSSTLTLSKADYEKHKVYACEVTHQGLSSPVTKSFNRGEC

SEQ ID NO: 43 - protein, 216 aa, synthetic construct
  REGION 1..216: note = Description of Artificial Sequence: Synthetic polypeptide
ALDIQLTQSPSFLSASVGDRVTITCRASQGIGNDLNWYQQKPGKAPKLLIYDASSLESGVPSRFSGSGSGTEFTLTISSLQPEDFATYYCQQADSWPLTFGGGTKVEIKRTVAAPSVFIFPPSDEQLKSGTASVVCLLNNFYPREAKVQWKVDNALQSGNSQESVTEQDSKDSTYSLSSTLTLSKADYEKHKVYACEVTHQGLSSPVTKSFNRGEC

SEQ ID NO: 44 - protein, 216 aa, synthetic construct
  REGION 1..216: note = Description of Artificial Sequence: Synthetic polypeptide
ALDIQLTQSPSFLSASVGDRVTITCRASQGISSYLAWYQQKPGKAPKLLIYAASTLQSGVPSRFSGSGSGTEFTLTISSLQPEDFATYYCQQLNSYPLTFGGGTKVEIKRTVAAPSVFIFPPSDEQLKSGTASVVCLLNNFYPREAKVQWKVDNALQSGNSQESVTEQDSKDSTYSLSSTLTLSKADYEKHKVYACEVTHQGLSSPVTKSFNRGEC

SEQ ID NO: 45 - protein, 218 aa, synthetic construct
  REGION 1..218: note = Description of Artificial Sequence: Synthetic polypeptide
ALQSALTQPASVSGSPGQSITISCTGTSSDVGGYNYVSWYQQHPGKAPKLIIYDVTKRPSGVSNRFSGSKSGNTASLTISGLQAEDEADYYCCSYTGTSNFVFGGGTKLTVLRQPKAAPSVTLFPPSSEELQANKATLVCLISDFYPGAVTVAWKADGSPVKAGVETTTPSKQSNNKYAASSYLSLTPEQWKSHKSYSCQVTHEGSTVEKTVAPTECS

SEQ ID NO: 46 - protein, 216 aa, synthetic construct
  REGION 1..216: note = Description of Artificial Sequence: Synthetic polypeptide
ALSYELMQPPSVSVSPGQTARITCSGDALPKQYAYWYQQKPGQAPVLVIYKDSERPSGIPERFSGSSSGTTVTLTISGVQAEDEADYYCQSADSSGTYVVFGGGTKLTVLRQPKAAPSVTLFPPSSEELQANKATLVCLISDFYPGAVTVAWKADGSPVKAGVETTTPSKQSNNKYAASSYLSLTPEQWKSHKSYSCQVTHEGSTVEKTVAPTECS

SEQ ID NO: 47 - protein, 218 aa, synthetic construct
  REGION 1..218: note = Description of Artificial Sequence: Synthetic polypeptide
ALQSALTQPASVSGSPGQSITISCTGTSSDVGGYNYVSWYQQHPGKAPKLMIYEVSNRPSGVSNRFSGSKSGNTASLTISGLQAEDEADYYCCSYTSTSNVVFGGGTKLTVLRQPKAAPSVTLFPPSSEELQANKATLVCLISDFYPGAVTVAWKADGSPVKAGVETTTPSKQSNNKYAASSYLSLTPEQWKSHKSYSCQVTHEGSTVEKTVAPTECS

SEQ ID NO: 48 - protein, 218 aa, synthetic construct
  REGION 1..218: note = Description of Artificial Sequence: Synthetic polypeptide
ALQSALTQPASVSGSPGQSITISCTGTSSDVGSYNYVSWYQQHPGKAPKLIIYEVSKRPSGVSNRFSGSKSGNTASLTISGLQAEDEADYYCSSYAGTSNVVFGGGTKLTVLRQPKAAPSVTLFPPSSEELQANKATLVCLISDFYPGAVTVAWKADGSPVKAGVETTTPSKQSNNKYAASSYLSLTPEQWKSHKSYSCQVTHEGSTVEKTVAPTECS

SEQ ID NO: 49 - protein, 216 aa, synthetic construct
  REGION 1..216: note = Description of Artificial Sequence: Synthetic polypeptide
ALSSELTQDPAVSVALGQTVRITCQGDSLRKKYVYWYQQKPGQAPVLVIYKDNNRPSGIPDRFSGSSSGNTASLTITGAQAEDEADYYCNSWDSSSAHYVFGGGTKLTVLRQPKAAPSVTLFPPSSEELQANKATLVCLISDFYPGAVTVAWKADGSPVKAGVETTTPSKQSNNKYAASSYLSLTPEQWKSHKSYSCQVTHEGSTVEKTVAPTECS

SEQ ID NO: 50 - protein, 218 aa, synthetic construct
  REGION 1..218: note = Description of Artificial Sequence: Synthetic polypeptide
ALQSALTQPASVSGSPGQSITISCTGTSSDVGSYNYVSWYQQHPGKAPKLMIYEVTNRPSGVSNRFSGSKSGNTASLTISGLQAEDEADYYCSSYASSSNLVFGGGTKLTVLRQPKAAPSVTLFPPSSEELQANKATLVCLISDFYPGAVTVAWKADGSPVKAGVETTTPSKQSNNKYAASSYLSLTPEQWKSHKSYSCQVTHEGSTVEKTVAPTECS

SEQ ID NO: 51 - protein, 218 aa, synthetic construct
  REGION 1..218: note = Description of Artificial Sequence: Synthetic polypeptide
ALQSALTQPASVSGSPGQSITISCTGTSSDVGGYNYVSWYQQHPGKAPKLIIYDVTNRPSGVSNRFSGSKSGNTASLTISGLQAEDEADYYCSSYTGSSSYVFGGGTKLTVLRQPKAAPSVTLFPPSSEELQANKATLVCLISDFYPGAVTVAWKADGSPVKAGVETTTPSKQSNNKYAASSYLSLTPEQWKSHKSYSCQVTHEGSTVEKTVAPTECS

SEQ ID NO: 52 - protein, 139 aa, synthetic construct
  REGION 1..139: note = Description of Artificial Sequence: Synthetic polypeptide
EVQLVESGGGLVKPGGSLRLSCAASGFTFSTYGMSWVRQAPGKGLEWVAYINNGSGYIYYADSVKGRFTISRDNAKNSLYLQMNSLRAEDTAVYYCARGQWWSGGDFDYWGQGTLVTVSSASTKGPSVFPLAPSSKSTS

SEQ ID NO: 53 - protein, 143 aa, synthetic construct
  REGION 1..143: note = Description of Artificial Sequence: Synthetic polypeptide
EVQLLESGGGLVQPGGSLRLSCAASGFTFSSYAMSWVRQAPGKGLEWVSAISGSGGSTYYADSVKGRFTISRDNSKNTLYLQMNSLRAEDTAVYYCARGYRASDSDYYGWMDYWGQGTLVTVSSASTKGPSVFPLAPSSKSTS

SEQ ID NO: 54 - protein, 138 aa, synthetic construct
  REGION 1..138: note = Description of Artificial Sequence: Synthetic polypeptide
QVQLVQSGAEVKKPGASVKVSCKASGYTFTGYYMHWVRQAPGQGLEWMGGINPNSGGTNYAQKFQGRVTMTRDTSISTAYMELSRLRSDDTAVYYCARRPAGPWALDYWGQGTLVTVSSASTKGPSVFPLAPSSKSTS

SEQ ID NO: 55 - protein, 136 aa, synthetic construct
  REGION 1..136: note = Description of Artificial Sequence: Synthetic polypeptide
QVQLVQSGAEVKKPGSSVKVSCKASGGTFTAYAINWVRQAPGQGLEWMGGINVGFGGANYAQKFQGRVTITADKSTSTAYMELSSLRSEDTAVYYCARDDYWTSVYWGQGTLVTVSSASTKGPSVFPLAPSSKSTS

SEQ ID NO: 56 - protein, 142 aa, synthetic construct
  REGION 1..142: note = Description of Artificial Sequence: Synthetic polypeptide
QVQLVQSGAEVKKPGASVKVSCKASGYTFSGYGMHWVRQAPGQGLEWMGWINPISGTATYAQKFQGRVTMTRDTSISTAYMELSRLRSDDTAVYYCAKDLIGWISHSYNGDYWGQGTLVTVSSASTKGPSVFPLAPSSKSTS

SEQ ID NO: 57 - protein, 138 aa, synthetic construct
  REGION 1..138: note = Description of Artificial Sequence: Synthetic polypeptide
EVQLVESGGGLVKPGGSLRLSCAASGFTFRSYEMHWVRQAPGKGLEWVASIKYDGANKNYADSVKGRFTISRDNAKNSLYLQMNSLRAEDTAVYYCARASPYGPSFDYWGQGTLVTVSSASTKGPSVFPLAPSSKSTS

SEQ ID NO: 58 - protein, 141 aa, synthetic construct
  REGION 1..141: note = Description of Artificial Sequence: Synthetic polypeptide
EVQLVESGGGLVKPGGSLRLSCAASGFTFSNFEMNWVRQAPGKGLEWVSGISSNGRYINYADSVKGRFTISRDNAKNSLYLQMNSLRAEDTAVYYCARVVDFDQDYNGFDYWGQGTLVTVSSASTKGPSVFPLAPSSKSTS

SEQ ID NO: 59 - protein, 138 aa, synthetic construct; identical to SEQ ID NO: 57
  REGION 1..138: note = Description of Artificial Sequence: Synthetic polypeptide

SEQ ID NO: 60 - protein, 138 aa, synthetic construct
  REGION 1..138: note = Description of Artificial Sequence: Synthetic polypeptide
QVQLVQSGAEVKKPGASVKVSCKASGYTFSAHGLNWVRQAPGQGLEWMGWINPITGTATYAQKFQGRVTMTRDTSISTAYMELSRLRSDDTAVYYCARGGWSNWGFDYWGQGTLVTVSSASTKGPSVFPLAPSSKSTS

SEQ ID NO: 61 - protein, 139 aa, synthetic construct
  REGION 1..139: note = Description of Artificial Sequence: Synthetic polypeptide
QVQLVQSGAEVKKPGSSVKVSCKASGGTFSNYAISWVRQAPGQGLEWMGWISPFSGGTNYAQKFQGRVTITADKSTSTAYMELSSLRSEDTAVYYCARGQWWYGDAFDYWGQGTLVTVSSASTKGPSVFPLAPSSKSTS

SEQ ID NO: 62 - protein, 142 aa, synthetic construct
  REGION 1..142: note = Description of Artificial Sequence: Synthetic polypeptide
QVQLVQSGAEVKKPGASVKVSCKASGYTFTGYYMHWVRQAPGQGLEWMGWINPNSGGTNYAQKFQGRVTMTRDTSISTAYMELSRLRSDDTAVYYCARGPIRSRGGKYGGDYWGQGTLVTVSSASTKGPSVFPLAPSSKSTS

SEQ ID NO: 63 - protein, 141 aa, synthetic construct
  REGION 1..141: note = Description of Artificial Sequence: Synthetic polypeptide
EVQLLESGGGLVQPGGSLRLSCAASGFTFSNYGMNWVRQAPGKGLEWVANIGYGGTNTYYADSVKGRFTISRDNSKNTLYLQMNSLRAEDTAVYYCAREAGYDRYGYGFDYWGQGTLVTVSSASTKGPSVFPLAPSSKSTS

SEQ ID NO: 64 - protein, 137 aa, synthetic construct
  REGION 1..137: note = Description of Artificial Sequence: Synthetic polypeptide
EVQLLESGGGLVQPGGSLRLSCAASGFTFSSYAMNWVRQAPGKGLEWVSVISGNSADKNYADSVKGRFTISRDNSKNTLYLQMNSLRAEDTAVYYCARGDGLNYLDYWGQGTLVTVSSASTKGPSVFPLAPSSKSTS

SEQ ID NO: 65 - protein, 140 aa, synthetic construct
  REGION 1..140: note = Description of Artificial Sequence: Synthetic polypeptide
EVQLLESGGGLVQPGGSLRLSCAASGFTFSSYGMNWVRQAPGKGLEWVATINYSGTSKYYADSVKGRFTISRDNSKNTLYLQMNSLRAEDTAVYYCARDRYKSYTYALDYWGQGTLVTVSSASTKGPSVFPLAPSSKSTS

SEQ ID NO: 66 - protein, 140 aa, synthetic construct
  REGION 1..140: note = Description of Artificial Sequence: Synthetic polypeptide
EVQLVESGGGLVKPGGSLRLSCAASGFTFSDYGMSWVRQAPGKGLEWVSGISWNGGTTNYADSVKGRFTISRDNAKNSLYLQMNSLRAEDTAVYYCARSGGAFYLSGLDYWGQGTLVTVSSASTKGPSVFPLAPSSKSTS

SEQ ID NO: 67 - protein, 136 aa, synthetic construct
  REGION 1..136: note = Description of Artificial Sequence: Synthetic polypeptide
QVQLVQSGAEVKKPGASVKVSCKASGYTFSSYGMSWVRQAPGQGLEWMGWINANSGGTSYAQKFQGRVTMTRDTSISTAYMELSRLRSDDTAVYYCARDDGGAYVYWGQGTLVTVSSASTKGPSVFPLAPSSKSTS

SEQ ID NO: 68 - protein, 180 aa, Homo sapiens; identical to SEQ ID NO: 12

SEQ ID NO: 69 - protein, 135 aa, Homo sapiens; identical to SEQ ID NO: 26